European Patent Application EP 4 144 762 A1, published March 8, 2023. Title: Structure and manufacturing method thereof, adsorbent using it, and method for purifying biological particles. Applicant: KANEKA CORPORATION. The sequence listing filed with the application follows.

SEQUENCE LISTING (4 sequences)

SEQ ID NO: 1 - protein, 263 aa, Artificial Sequence
  anti AAV2-scFv
MDASDVQLQESGPDLVKPSQSLSLTCTVTGYSITSGYTWHWIRQFPGNKQEWMGYIHFSGYTNYNPSLKSRVSITRDTSKNQFFLHLNSVTTEDTATYYCARGDYGYEWFTYWGQGTLVTVSAGGGGSGGGGSGGGGSIQMTQSSSSFSVSLGDRVTITCKASEDIHNRLAWYKQKPGNAPRLLISGATSLETGVPSRFSGSGSGKDYTLSITSLQNEDVATYYCQQYWIGPFTFGSGTNLEIKRADAAPTVAAAIEHHHHHH

SEQ ID NO: 2 - DNA, 766 bp, Artificial Sequence
  anti AAV2-scFv
ccatggatgcctcggatgttcagctgcaagaaagcggccctgacctggtcaaaccgtcacaaagcttgtccctgacatgcaccgtaaccgggtattccattaccagcggctatacctggcattggattcgccagtttccggggaataagcaggaatggatgggctatatccactttagtggctacacgaactataacccctcgctgaaatcccgtgtcagtatcacacgcgatacgtcaaagaaccagttcttcctccatctgaactcggttaccacagaagatactgcgacgtattattgtgcccgtggggactatggttatgaatggttcacgtattggggtcaaggcacgctggtgactgtaagcgctggtggaggtggctctggtggtggcggtagcggtggcggtggctcgatccagatgacgcaaagcagttctagcttcagcgtgtctcttggcgatcgtgtcaccatcacttgcaaagcgtctgaggacattcacaatcgccttgcctggtacaaacagaaaccagggaatgcaccacgcttactcattagtggcgcgacgtcactggaaaccggtgtgccgtcacgcttttcgggaagtggatctgggaaagactacactttgagcattacctccttacagaatgaggatgtggcgacctactactgtcaacagtactggattggcccgtttacctttggctccggtaccaacctggaaatcaaacgggctgatgctgcgccgacagttgcggccgc

SEQ ID NO: 3 - protein, 136 aa, Artificial Sequence
  anti AAV2-VHH
QVQLVESGGGLVQAGGSLRLSCAASGRTFSSYAMGWFRQAPGKEREIVASISWNGGSTDYADSVKGRFTISRDNAKNTVYLQMNSLKPEDTAVYYCAADSTNWVFYDYWGQGTQVTVSSEPKTPKPQTSAHHHHHH

SEQ ID NO: 4 - DNA, 558 bp, Artificial Sequence
  anti AAV2-VHH
tctagaaataattttgtttaactttaagaaggagatatacatatgaaatacctgctgccgaccgctgctgctggtctgctgctcctcgcggcccagccggccatggctcaggtgcagctcgtggagtctgggggaggcctggttcaggctggtgggtcattacgcctgtcttgcgcagcatctggtcgtacgttttcgtcctatgcgatgggctggtttcgtcaagctccaggcaaagaacgcgagattgttgcgagcatctcctggaatggtggcagtaccgactatgccgatagcgtcaaaggacggttcaccattagtcgcgataacgccaagaacacggtgtacttgcagatgaacagcctgaaaccggaagatactgcggtatactattgtgccgcggattcgaccaattgggtgttctacgactattggggtcaagggacacaggtcaccgtctcctcagaaccgaaaacgccaaaaccgcagacatcggcccatcatcaccaccatcactaataactgcaggcttgcaagcttctgctgccaccgctgagc